European Patent Application EP 4 548 929 A1, published May 7, 2025. Title: Pharmaceutical composition comprising mixture of antibodies of anti-CTLA4 and anti-PD1, and therapeutic use thereof. Applicant: QILU PHARMACEUTICAL CO., LTD. Application CN. The sequence listing filed with the application follows.

SEQUENCE LISTING (20 sequences)

SEQ ID NO: 1 - protein, 5 aa, synthetic construct
SYGMH

SEQ ID NO: 2 - protein, 17 aa, synthetic construct
VIWYKPSEKDYADSAKG

SEQ ID NO: 3 - protein, 9 aa, synthetic construct
GGLLGYFDY

SEQ ID NO: 4 - protein, 11 aa, synthetic construct
RASQSINSYLA

SEQ ID NO: 5 - protein, 7 aa, synthetic construct
GVSSRAT

SEQ ID NO: 6 - protein, 9 aa, synthetic construct
QQYGRYPFT

SEQ ID NO: 7 - protein, 118 aa, synthetic construct
QVQLVESGGGVVEPGRSLRLSCAASGFTFSSYGMHWVRQAPGKGLEWVAVIWYKPSEKDYADSAKGRFTISRDNSKNTLYLQMNSLRAEDTAVYYCARGGLLGYFDYWGQGTLVTVSS

SEQ ID NO: 8 - protein, 107 aa, synthetic construct
EIVLTQSPGTLSLSPGERATLSCRASQSINSYLAWYQQKPGQAPRPLIYGVSSRATGIPDRFSGSGSGTDFTLTISRLEPEDFAVYYCQQYGRYPFTFGPGTKVDIK

SEQ ID NO: 9 - protein, 5 aa, synthetic construct
NYWIH

SEQ ID NO: 10 - protein, 17 aa, synthetic construct
EIDPYDSYTNYNQKFKG

SEQ ID NO: 11 - protein, 10 aa, synthetic construct
PGFTYGGMDF

SEQ ID NO: 12 - protein, 17 aa, synthetic construct
KSSQSLFNSGNQKNYLA

SEQ ID NO: 13 - protein, 7 aa, synthetic construct
GASTRDS

SEQ ID NO: 14 - protein, 9 aa, synthetic construct
QNDHYYPYT

SEQ ID NO: 15 - protein, 119 aa, synthetic construct
QVQLVQSGAEVKKPGASVKVSCKASGYTFTNYWIHWVRQAPGQGLEWMGEIDPYDSYTNYNQKFKGRVTMTVDKSTSTVYMELSSLRSEDTAVYYCARPGFTYGGMDFWGQGTLVTVSS

SEQ ID NO: 16 - protein, 113 aa, synthetic construct
DIQMTQSPSSLSASVGDRVTITCKSSQSLFNSGNQKNYLAWYQQKPGKVPKLLIYGASTRDSGVPYRFSGSGSGTDFTLTISSLQPEDVATYYCQNDHYYPYTFGGGTKVEIK

SEQ ID NO: 17 - protein, 448 aa, synthetic construct
QVQLVESGGGVVEPGRSLRLSCAASGFTFSSYGMHWVRQAPGKGLEWVAVIWYKPSEKDYADSAKGRFTISRDNSKNTLYLQMNSLRAEDTAVYYCARGGLLGYFDYWGQGTLVTVSSASTKGPSVFPLAPSSKSTSGGTAALGCLVDDYFPEPVTVSWNSGALTSGVHTCPACLQSSGLYSLSSVVTVPSSSLGTQTYICNVNHKPSNTKVDKKVEPKSGDKTHTCPPCPAPELLGGPSVFLFPPKPKDTLMISKTPEVTCVVVDVSHEDPEVKFNWYVDGVEVHNAKTKPREEQYNSTYRVVSVLTVLHQDWLNGKEYKCKVSNKALPAPIEKTISKAKGQPREPQVYTLPPSREEMTKNQVSLTCLVKGFYPSDIAVEWESNGQPENNYKTTPPVLRSDGSFFLYSELTVDKSRWQQGNVFSCSVMHEALHNHYTQKSLSLSPGK

SEQ ID NO: 18 - protein, 214 aa, synthetic construct
EIVLTQSPGTLSLSPGERATLSCRASQSINSYLAWYQQKPGQAPRPLIYGVSSRATGIPDRFSGSGSGTDFTLTISRLEPEDFAVYYCQQYGRYPFTFGPGTKVDIKRTVAAPSVFIFPPSDEQLKSGTAKVVCLLNNFYPREAKVQWKVDNALQSGNSCECVTEQDSKDSTYSLSSTLTLSKADYEKHKVYACEVTHQGLSSPVTKSFNRGES

SEQ ID NO: 19 - protein, 446 aa, synthetic construct
QVQLVQSGAEVKKPGASVKVSCKASGYTFTNYWIHWVRQAPGQGLEWMGEIDPYDSYTNYNQKFKGRVTMTVDKSTSTVYMELSSLRSEDTAVYYCARPGFTYGGMDFWGQGTLVTVSSASTKGPSVFPLAPCSRSTSESTAALGCLVKDYFPEPVTVSWNSGALTSGVHTFPAVLQSSGLYSLSSVVTVPSSSLGTKTYTCNVDHKPSNTKVDKRVESKYGPPCPPCPAPEFLGGPSVFLFPPKPKDTLMISRTPEVTCVVVDVSQEDPEVQFNWYVDGVEVHNAKTKPREEQFNSTYRVVSVLTVLHQDWLNGKEYKCKVSNKGLPSSIEKTISKAKGQPREPQVYTLPPSQEEMTKNQVSLTCLVKGFYPSDIAVEWESNGQPENNYKTTPPVLDSDGSFFLYSRLTVDKSRWQEGNVFSCSVMHEALHNHYTQKSLSLSLGK

SEQ ID NO: 20 - protein, 220 aa, synthetic construct
DIQMTQSPSSLSASVGDRVTITCKSSQSLFNSGNQKNYLAWYQQKPGKVPKLLIYGASTRDSGVPYRFSGSGSGTDFTLTISSLQPEDVATYYCQNDHYYPYTFGGGTKVEIKRTVAAPSVFIFPPSDEQLKSGTASVVCLLNNFYPREAKVQWKVDNALQSGNSQESVTEQDSKDSTYSLSSTLTLSKADYEKHKVYACEVTHQGLSSPVTKSFNRGEC